European Patent Specification EP 3 943 508 B1, published January 10, 2024. Title: DUAL FUNCTION ANTIBODIES SPECIFIC TO GLYCOSYLATED PD-L1 AND METHODS OF USE THEREOF. Applicant: STCUBE, INC. BOARD OF REGENTS, THE UNIVERSITY OF TEXAS SYSTEM. Application 17715372.3. The sequence listing filed with the application follows.

SEQUENCE LISTING (100 sequences)

SEQ ID NO: 1 - protein, 290 aa, Homo sapiens
MRIFAVFIFMTYWHLLNAFTVTVPKDLYVVEYGSNMTIECKFPVEKQLDLAALIVYWEMEDKNIIQFVHGEEDLKVQHSSYRQRARLLKDQLSLGNAALQITDVKLQDAGVYRCMISYGGADYKRITVKVNAPYNKINQRILVVDPVTSEHELTCQAEGYPKAEVIWTSSDHQVLSGKTTTTNSKREEKLFNVTSTLRINTTTNEIFYCTFRRLDPEENHTAELVIPELPLAHPPNERTHLVILGAILLCLGVALTFIFRLRKGRMMDVKKCGIQDTNSKKQSDTHLEET

SEQ ID NO: 2 - DNA, 350 bp, Artificial Sequence
  Description of Artificial Sequence: Synthetic polynucleotide
aagtgcagctggtggagtctgggggagccttagtgaagcctggagggtccctgaaactctcctgtgcagcctctggattcactttcagtaactctgccatgtcttgggttcgccagactccagagaagaggctggagtgggtcgcaaccattagtagtgctggtagttatacctactatccagacagtgtgaagggtcgattcaccatctccagagacaatgccaagaacaccctgtacctgcaaatgagcagtctgaggtctgaggacacggccttgtattactgtacaagacattatgattactactttgactactggggccaaggcgccactctcacagtctcctca

SEQ ID NO: 3 - protein, 117 aa, Artificial Sequence
  Description of Artificial Sequence: Synthetic polypeptide
EVQLVESGGALVKPGGSLKLSCAASGFTFSNSAMSWVRQTPEKRLEWVATISSAGSYTYYPDSVKGRFTISRDNAKNTLYLQMSSLRSEDTALYYCTRHYDYYFDYWGQGATLTVSS

SEQ ID NO: 4 - protein, 7 aa, Artificial Sequence
  Description of Artificial Sequence: Synthetic peptide
GFTFSNS

SEQ ID NO: 5 - protein, 5 aa, Artificial Sequence
  Description of Artificial Sequence: Synthetic peptide
NSAMS

SEQ ID NO: 6 - protein, 6 aa, Artificial Sequence
  Description of Artificial Sequence: Synthetic peptide
SSGGSY

SEQ ID NO: 7 - protein, 17 aa, Artificial Sequence
  Description of Artificial Sequence: Synthetic peptide
TISSAGSYTYYPDSVKG

SEQ ID NO: 8 - protein, 10 aa, Artificial Sequence
  Description of Artificial Sequence: Synthetic peptide
TRHYDYYFDY

SEQ ID NO: 9 - protein, 10 aa, Artificial Sequence
  Description of Artificial Sequence: Synthetic peptide
TRHYDYYFDY

SEQ ID NO: 10 - DNA, 319 bp, Artificial Sequence
  Description of Artificial Sequence: Synthetic polynucleotide
caaattgttctcacccagtctccagcaatcatgtctgcatctccaggggagaaggtcaccttgacctgcagtgccagctcaagtgtaagttacatgcattggtaccagcagaagccaggatcctcccccagactcgtgatttatgacacatccaacctggcttctggagtccctgttcgcttcagtggcagtgggtctgggacctcttactctctcacagtcagccgaatggaggctgaagatgctgccacttattactgccagcagtggagtgatcacccgctcacgttcggtgctgggaccaagctggagctgaaac

SEQ ID NO: 11 - protein, 106 aa, Artificial Sequence
  Description of Artificial Sequence: Synthetic polypeptide
QIVLTQSPAIMSASPGEKVTLTCSASSSVSYMHWYQQKPGSSPRLVIYDTSNLASGVPVRFSGSGSGTSYSLTVSRMEAEDAATYYCQQWSDHPLTFGAGTKLELK

SEQ ID NO: 12 - protein, 10 aa, Artificial Sequence
  Description of Artificial Sequence: Synthetic peptide
SASSSVSYMH

SEQ ID NO: 13 - protein, 10 aa, Artificial Sequence
  Description of Artificial Sequence: Synthetic peptide
SASSSVSYMH

SEQ ID NO: 14 - protein, 7 aa, Artificial Sequence
  Description of Artificial Sequence: Synthetic peptide
DTSNLAS

SEQ ID NO: 15 - protein, 7 aa, Artificial Sequence
  Description of Artificial Sequence: Synthetic peptide
DTSNLAS

SEQ ID NO: 16 - protein, 9 aa, Artificial Sequence
  Description of Artificial Sequence: Synthetic peptide
QQWSDHPLT

SEQ ID NO: 17 - protein, 9 aa, Artificial Sequence
  Description of Artificial Sequence: Synthetic peptide
QQWSDHPLT

SEQ ID NO: 18 - DNA, 357 bp, Artificial Sequence
  Description of Artificial Sequence: Synthetic polynucleotide
gaagtgatgctggtggagtctgggggagccttagtgaagcctggagggtccctgaaactctcctgtgcagcttctggattcagtttgagtaactatgtcatgtcttgggttcgccagactccagagaagaggctggagtgggtcgcaaccattagtagtggtggtaggtatatctactatacagacagtgtgaagggtcgattcaccatctccagggacaatgccaggaacaccctgtacctgcaaatgagcagtctgaggtctgaggacacggccatgtattattgtgcaagagacggtagtaccttgtactactttgactattggggccaaggcaccactctcacagtctcctca

SEQ ID NO: 19 - protein, 119 aa, Artificial Sequence
  Description of Artificial Sequence: Synthetic polypeptide
EVMLVESGGALVKPGGSLKLSCAASGFSLSNYVMSWVRQTPEKRLEWVATISSGGRYIYYTDSVKGRFTISRDNARNTLYLQMSSLRSEDTAMYYCARDGSTLYYFDYWGQGTTLTVSS

SEQ ID NO: 20 - protein, 7 aa, Artificial Sequence
  Description of Artificial Sequence: Synthetic peptide
GFSLSNY

SEQ ID NO: 21 - protein, 5 aa, Artificial Sequence
  Description of Artificial Sequence: Synthetic peptide
NYVMS

SEQ ID NO: 22 - protein, 6 aa, Artificial Sequence
  Description of Artificial Sequence: Synthetic peptide
SSGGRY

SEQ ID NO: 23 - protein, 17 aa, Artificial Sequence
  Description of Artificial Sequence: Synthetic peptide
TISSGGRYIYYTDSVKG

SEQ ID NO: 24 - protein, 10 aa, Artificial Sequence
  Description of Artificial Sequence: Synthetic peptide
DGSTLYYFDY

SEQ ID NO: 25 - protein, 10 aa, Artificial Sequence
  Description of Artificial Sequence: Synthetic peptide
DGSTLYYFDY

SEQ ID NO: 26 - DNA, 378 bp, Artificial Sequence
  Description of Artificial Sequence: Synthetic polynucleotide
caagtgcagattttcagcttcctgctaatcagtgcctcagtcatactgtccagaggacaaactgttctcacccagtctccagcaatcatgtctgcatctccaggggagaaggtcaccatgacctgcagtgccagctcaagtgtagattacatgtactggtaccagcagaagccaggatcctcccccagactcctgatttatgacacatccaacctggcttctggagtccctgttcgcttcagtggcagtgggtctgggacctcttactctctcacaatcagccgaatggaggctgaagatgctgccacttattactgccagcagtggagtagttccccacccatcacgttcggtactgggaccaaggtggagctgaaa

SEQ ID NO: 27 - protein, 126 aa, Artificial Sequence
  Description of Artificial Sequence: Synthetic polypeptide
QVQIFSFLLISASVILSRGQTVLTQSPAIMSASPGEKVTMTCSASSSVDYMYWYQQKPGSSPRLLIYDTSNLASGVPVRFSGSGSGTSYSLTISRMEAEDAATYYCQQWSSSPPITFGTGTKVELK

SEQ ID NO: 28 - protein, 10 aa, Artificial Sequence
  Description of Artificial Sequence: Synthetic peptide
SASSSVDYMY

SEQ ID NO: 29 - protein, 10 aa, Artificial Sequence
  Description of Artificial Sequence: Synthetic peptide
SASSSVDYMY

SEQ ID NO: 30 - protein, 7 aa, Artificial Sequence
  Description of Artificial Sequence: Synthetic peptide
DTSNLAS

SEQ ID NO: 31 - protein, 7 aa, Artificial Sequence
  Description of Artificial Sequence: Synthetic peptide
DTSNLAS

SEQ ID NO: 32 - protein, 10 aa, Artificial Sequence
  Description of Artificial Sequence: Synthetic peptide
QQWSSSPPIT

SEQ ID NO: 33 - protein, 10 aa, Artificial Sequence
  Description of Artificial Sequence: Synthetic peptide
QQWSSSPPIT

SEQ ID NO: 34 - DNA, 19 bp, Artificial Sequence
  Description of Artificial Sequence: Synthetic oligonucleotide
tcaattgtcatattgctac

SEQ ID NO: 35 - DNA, 19 bp, Artificial Sequence
  Description of Artificial Sequence: Synthetic oligonucleotide
ttgactccatctttcttca

SEQ ID NO: 36 - DNA, 39 bp, Artificial Sequence
  Description of Artificial Sequence: Synthetic primer
gtggtagagtatggtagccaaatgacaattgaatgcaaa

SEQ ID NO: 37 - DNA, 39 bp, Artificial Sequence
  Description of Artificial Sequence: Synthetic primer
tttgcattcaattgtcatttggctaccatactctaccac

SEQ ID NO: 38 - DNA, 37 bp, Artificial Sequence
  Description of Artificial Sequence: Synthetic primer
gagaggagaagcttttccaggtgaccagcacactgag

SEQ ID NO: 39 - DNA, 37 bp, Artificial Sequence
  Description of Artificial Sequence: Synthetic primer
ctcagtgtgctggtcacctggaaaagcttctcctctc

SEQ ID NO: 40 - DNA, 39 bp, Artificial Sequence
  Description of Artificial Sequence: Synthetic primer
gaccagcacactgagaatccagacaacaactaatgagat

SEQ ID NO: 41 - DNA, 39 bp, Artificial Sequence
  Description of Artificial Sequence: Synthetic primer
atctcattagttgttgtctggattctcagtgtgctggtc

SEQ ID NO: 42 - DNA, 40 bp, Artificial Sequence
  Description of Artificial Sequence: Synthetic primer
gagagaggagaagcttttccaagtgaccagcacactgaga

SEQ ID NO: 43 - DNA, 40 bp, Artificial Sequence
  Description of Artificial Sequence: Synthetic primer
tctcagtgtgctggtcacttggaaaagcttctcctctctc

SEQ ID NO: 44 - DNA, 22 bp, Artificial Sequence
  Description of Artificial Sequence: Synthetic primer
gcataacgaacctaaccctcag

SEQ ID NO: 45 - DNA, 20 bp, Artificial Sequence
  Description of Artificial Sequence: Synthetic primer
gcccaatgtccactgtgata

SEQ ID NO: 46 - DNA, 19 bp, Artificial Sequence
  Description of Artificial Sequence: Synthetic primer
gtaacctcagtcacctgcc

SEQ ID NO: 47 - DNA, 20 bp, Artificial Sequence
  Description of Artificial Sequence: Synthetic primer
attccgctccacaatctctg

SEQ ID NO: 48 - DNA, 20 bp, Artificial Sequence
  Description of Artificial Sequence: Synthetic primer
tcttcaacctcacgctcaag

SEQ ID NO: 49 - DNA, 21 bp, Artificial Sequence
  Description of Artificial Sequence: Synthetic primer
gtgtgcaaagacgtcatcatc

SEQ ID NO: 50 - DNA, 23 bp, Artificial Sequence
  Description of Artificial Sequence: Synthetic primer
caccatcaccctcctttctattc

SEQ ID NO: 51 - DNA, 22 bp, Artificial Sequence
  Description of Artificial Sequence: Synthetic primer
gaacaacaggtctgggatttct

SEQ ID NO: 52 - DNA, 19 bp, Artificial Sequence
  Description of Artificial Sequence: Synthetic primer
gccttttgccatcgacatg

SEQ ID NO: 53 - DNA, 21 bp, Artificial Sequence
  Description of Artificial Sequence: Synthetic primer
agtcagattcttgcatccctg

SEQ ID NO: 54 - DNA, 22 bp, Artificial Sequence
  Description of Artificial Sequence: Synthetic primer
caaggagagcattaggaccaag

SEQ ID NO: 55 - DNA, 21 bp, Artificial Sequence
  Description of Artificial Sequence: Synthetic primer
ccccattaaacctcaggactg

SEQ ID NO: 56 - DNA, 20 bp, Artificial Sequence
  Description of Artificial Sequence: Synthetic primer
tcgtcatggtgtggtattcc

SEQ ID NO: 57 - DNA, 19 bp, Artificial Sequence
  Description of Artificial Sequence: Synthetic primer
caggaagatgggctgatcc

SEQ ID NO: 58 - DNA, 20 bp, Artificial Sequence
  Description of Artificial Sequence: Synthetic primer
gaccgcactcatcttacacc

SEQ ID NO: 59 - DNA, 21 bp, Artificial Sequence
  Description of Artificial Sequence: Synthetic primer
ggaggttggctgaaggaatac

SEQ ID NO: 60 - DNA, 19 bp, Artificial Sequence
  Description of Artificial Sequence: Synthetic primer
tcccctgctttaaccatcg

SEQ ID NO: 61 - DNA, 21 bp, Artificial Sequence
  Description of Artificial Sequence: Synthetic primer
ttgtcacctatactggcgttg

SEQ ID NO: 62 - DNA, 21 bp, Artificial Sequence
  Description of Artificial Sequence: Synthetic primer
ctgagtgatggaacgagtgag

SEQ ID NO: 63 - DNA, 21 bp, Artificial Sequence
  Description of Artificial Sequence: Synthetic primer
tagagatgaccagatgcaacg

SEQ ID NO: 64 - DNA, 21 bp, Artificial Sequence
  Description of Artificial Sequence: Synthetic primer
gagtccaacttcacggcttat

SEQ ID NO: 65 - DNA, 21 bp, Artificial Sequence
  Description of Artificial Sequence: Synthetic primer
agtggtccaggaagacataga

SEQ ID NO: 66 - DNA, 21 bp, Artificial Sequence
  Description of Artificial Sequence: Synthetic primer
tgtgagggaaagatcaagtgg

SEQ ID NO: 67 - DNA, 22 bp, Artificial Sequence
  Description of Artificial Sequence: Synthetic primer
gctctccaaggtaaatgaggac

SEQ ID NO: 68 - DNA, 20 bp, Artificial Sequence
  Description of Artificial Sequence: Synthetic primer
ccactgagttcgtcaagagg

SEQ ID NO: 69 - DNA, 20 bp, Artificial Sequence
  Description of Artificial Sequence: Synthetic primer
acttccttgccatctgtcac

SEQ ID NO: 70 - DNA, 20 bp, Artificial Sequence
  Description of Artificial Sequence: Synthetic primer
tggctcgctgataagttctg

SEQ ID NO: 71 - DNA, 21 bp, Artificial Sequence
  Description of Artificial Sequence: Synthetic primer
gtgagtctggtttgggagaag

SEQ ID NO: 72 - DNA, 21 bp, Artificial Sequence
  Description of Artificial Sequence: Synthetic primer
gcaaagacctgtacgccaaca

SEQ ID NO: 73 - DNA, 18 bp, Artificial Sequence
  Description of Artificial Sequence: Synthetic primer
tgcatcctgtcggcaatg

SEQ ID NO: 74 - protein, 53 aa, Artificial Sequence
  Description of Artificial Sequence: Synthetic consensus sequence
  MOD_RES (21)..(21): Ile, Met or Leu
  MOD_RES (32)..(32): Asp or Asn
AFTITVPKDLYVVEYGSNVTXECRFPVEKQLXLLALVVYWEMEDKKIIQFVNG

SEQ ID NO: 75 - protein, 53 aa, Homo sapiens
AFTVTVPKDLYVVEYGSNMTIECKFPVEKQLDLAALIVYWEMEDKNIIQFVHG

SEQ ID NO: 76 - protein, 53 aa, Mus musculus
AFTITAPKDLYVVEYGSNVTMECRFPVERELDLLALVVYWEKEDEQVIQFVAG

SEQ ID NO: 77 - protein, 53 aa, Rattus norvegicus
AFTITAPKDLYVVEYGSNVTMECRFPVEQKLDLLALVVYWEKEDKEVIQFVEG

SEQ ID NO: 78 - protein, 53 aa, Bos taurus
AFTITVSKDLYVVEYGSNVTLECRFPVDKQLNLLVLVVYWEMEDKKIIQFVNG

SEQ ID NO: 79 - protein, 53 aa, Sus scrofa
AFTITVPKDMYEVEYGSNVTLECRFPVDKQLNLLALVVYWEMKDKKIIQFVNG

SEQ ID NO: 80 - protein, 53 aa, Equus caballus
AFTITVTKDLYVVDYGSNVTIECKFPVEEPLNLAALIVYWEMENKKIIQFVNG

SEQ ID NO: 81 - protein, 23 aa, Homo sapiens
KDLYVVEYGSNMTIECKFPVEKQ

SEQ ID NO: 82 - protein, 11 aa, Homo sapiens
KLFNVTSTLRI

SEQ ID NO: 83 - protein, 16 aa, Homo sapiens
RINTTTNEIFYCTFRR

SEQ ID NO: 84 - protein, 28 aa, Homo sapiens
RRLDPEENHTAELVIPELPLAHPPNERT

SEQ ID NO: 85 - protein, 61 aa, Homo sapiens
VHGEEDLKVQHSSYRQRARLLKDQLSLGNAALQITDVKLQDAGVYRCMISYGGADYKRITV

SEQ ID NO: 86 - protein, 21 aa, Homo sapiens
DAGVYRCMISYGGADYKRITV

SEQ ID NO: 87 - DNA, 408 bp, Artificial Sequence
  Description of Artificial Sequence: Synthetic polynucleotide
atgaacttgtggctcagcttggttttccttgtccttgttttaaaaggtgtccagtgtgaagtgcagctggtggagtctgggggagccttagtgaagcctggagggtccctgaaactctcctgtgcagcctctggattcactttcagtaactctgccatgtcttgggttcgccagactccagagaagaggctggagtgggtcgcaaccattagtagtgctggtagttatacctactatccagacagtgtgaagggtcgattcaccatctccagagacaatgccaagaacaccctgtacctgcaaatgagcagtctgaggtctgaggacacggccttgtattactgtacaagacattatgattactactttgactactggggccaaggcgccactctcacagtctcctca

SEQ ID NO: 88 - protein, 136 aa, Artificial Sequence
  Description of Artificial Sequence: Synthetic polypeptide
MNLWLSLVFLVLVLKGVQCEVQLVESGGALVKPGGSLKLSCAASGFTFSNSAMSWVRQTPEKRLEWVATISSAGSYTYYPDSVKGRFTISRDNAKNTLYLQMSSLRSEDTALYYCTRHYDYYFDYWGQGATLTVSS

SEQ ID NO: 89 - DNA, 385 bp, Artificial Sequence
  Description of Artificial Sequence: Synthetic polynucleotide
atggattttcaagtgcagattttcagcttcctgctaatcagtgcctcagtcatactgtccagaggacaaattgttctcacccagtctccagcaatcatgtctgcatctccaggggagaaggtcaccttgacctgcagtgccagctcaagtgtaagttacatgcattggtaccagcagaagccaggatcctcccccagactcgtgatttatgacacatccaacctggcttctggagtccctgttcgcttcagtggcagtgggtctgggacctcttactctctcacagtcagccgaatggaggctgaagatgctgccacttattactgccagcagtggagtgatcacccgctcacgttcggtgctgggaccaagctggagctgaaac

SEQ ID NO: 90 - protein, 128 aa, Artificial Sequence
  Description of Artificial Sequence: Synthetic polypeptide
MDFQVQIFSFLLISASVILSRGQIVLTQSPAIMSASPGEKVTLTCSASSSVSYMHWYQQKPGSSPRLVIYDTSNLASGVPVRFSGSGSGTSYSLTVSRMEAEDAATYYCQQWSDHPLTFGAGTKLELK

SEQ ID NO: 91 - DNA, 414 bp, Artificial Sequence
  Description of Artificial Sequence: Synthetic polynucleotide
atgaacttcgggctcagcttgattttccttgtccttattttaaaaggtgtccagtgtgaagtgatgctggtggagtctgggggagccttagtgaagcctggagggtccctgaaactctcctgtgcagcttctggattcagtttgagtaactatgtcatgtcttgggttcgccagactccagagaagaggctggagtgggtcgcaaccattagtagtggtggtaggtatatctactatacagacagtgtgaagggtcgattcaccatctccagggacaatgccaggaacaccctgtacctgcaaatgagcagtctgaggtctgaggacacggccatgtattattgtgcaagagacggtagtaccttgtactactttgactattggggccaaggcaccactctcacagtctcctca

SEQ ID NO: 92 - protein, 138 aa, Artificial Sequence
  Description of Artificial Sequence: Synthetic polypeptide
MNFGLSLIFLVLILKGVQCEVMLVESGGALVKPGGSLKLSCAASGFSLSNYVMSWVRQTPEKRLEWVATISSGGRYIYYTDSVKGRFTISRDNARNTLYLQMSSLRSEDTAMYYCARDGSTLYYFDYWGQGTTLTVSS

SEQ ID NO: 93 - protein, 6 aa, Artificial Sequence
  Description of Artificial Sequence: Synthetic 6xHis tag
HHHHHH

SEQ ID NO: 94 - protein, 53 aa, Artificial Sequence
  Description of Artificial Sequence: Synthetic consensus sequence
  MOD_RES (12)..(12): Ile or Val
  MOD_RES (44)..(44): Leu, Ala, Val or Tyr
  MOD_RES (45)..(45): Ala, Thr, Pro, Leu, Val or Ile
  MOD_RES (46)..(46): His, Arg, Asp or Val
  MOD_RES (48)..(48): Pro or Ala
EKLFNVTSTLRXNATANEIFYCTFRRLGPEENHTAELVIPELPXXXPXNKRTH

SEQ ID NO: 95 - protein, 53 aa, Homo sapiens
EKLFNVTSTLRINTTTNEIFYCTFRRLDPEENHTAELVIPELPLAHPPNERTH

SEQ ID NO: 96 - protein, 53 aa, Mus musculus
GMLLNVTSSLRVNATANDVFYCTFWRSQPGQNHTAELIIPELPATHPPQNRTH

SEQ ID NO: 97 - protein, 53 aa, Rattus norvegicus
EKLLNVTSVLRVNATANDVFHCTFWRVHSGENHTAELIIPELPVPRLPHNRTH

SEQ ID NO: 98 - protein, 52 aa, Bos taurus
EKLFNVTSTLRINTTADKIFYCTFRRLGHEENNTAELVIPEPYLDPAKKRNH

SEQ ID NO: 99 - protein, 52 aa, Sus scrofa
EKLFNVTSTLRVNATTNEIFYCTFRRLGPEENSTAVLVIPEPYVDPARKRTH

SEQ ID NO: 100 - protein, 52 aa, Equus caballus
EKLFNVTSTLRINATANEIFYCTFRRSGLEENSTAELVIPEPLIVPANKRTH